European Patent Specification EP 3 630 969 B1, published June 7, 2023. Title: OPTIMIZATION OF THE EXPRESSION OF SERINE PROTEASES IN HOST CELLS. Applicant: B.R.A.I.N. Biotechnology Research And Information Network AG. The sequence listing filed with the application follows.

SEQUENCE LISTING (12 sequences)

SEQ ID NO: 1 - protein, 58 aa, Bos taurus [sequence omitted]

SEQ ID NO: 2 - DNA, 177 bp, Artificial Sequence
  Codon-optimized nucleotide sequence of aprotinin
agaccagacttctgtttggaaccaccatacactggtccatgtaaggctagaatcatcagatacttctacaacgctaaggctggtttgtgtcagactttcgtttacggtggttgtagagctaagagaaacaacttcaagtccgctgaggactgtatgagaacttgtggtggtgcttaa

SEQ ID NO: 3 - protein, 254 aa, Lucilia sericata
MFRFVALFAFVSCALAGAIPNDLDGRIVNGVDTTIQAHPYQVSLQTNNGFHFCGGSIISEDIIVTAAHCMQSYKAYQFKVRLGSTEYDNGGELVAVKSFKYHEGYNPETMVNDVAVIKLATPVRESSKVRYVKLAEKTPATGTPAVVTGWGSKCFLFCQTAPKVLQKVEVDIVDEKTCASSEYKYGDDIKETMLCAYAVKKDACQGDSGGPLVANNKLVGVVSWGKGCALAGYPGVYCDVATVRSWIEKTAKSL

SEQ ID NO: 4 - protein, 238 aa, Lucilia sericata
GAIPNDLDGRIVNGVDTTIQAHPYQVSLQTNNGFHFCGGSIISEDIIVTAAHCMQSYKAYQFKVRLGSTEYDNGGELVAVKSFKYHEGYNPETMVNDVAVIKLATPVRESSKVRYVKLAEKTPATGTPAVVTGWGSKCFLFCQTAPKVLQKVEVDIVDEKTCASSEYKYGDDIKETMLCAYAVKKDACQGDSGGPLVANNKLVGVVSWGKGCALAGYPGVYCDVATVRSWIEKTAKSL

SEQ ID NO: 5 - protein, 228 aa, Lucilia sericata
IVNGVDTTIQAHPYQVSLQTNNGFHFCGGSIISEDIIVTAAHCMQSYKAYQFKVRLGSTEYDNGGELVAVKSFKYHEGYNPETMVNDVAVIKLATPVRESSKVRYVKLAEKTPATGTPAVVTGWGSKCFLFCQTAPKVLQKVEVDIVDEKTCASSEYKYGDDIKETMLCAYAVKKDACQGDSGGPLVANNKLVGVVSWGKGCALAGYPGVYCDVATVRSWIEKTAKSL

SEQ ID NO: 6 - DNA, 765 bp, Lucilia sericata
atgttccggtttgtagctctattcgctttcgttagctgtgccttggcgggcgctattcccaatgatttggatggccgcattgtcaatggtgtggataccaccattcaggcccatccctatcaggtttctttgcaaaccaacaatggtttccatttctgcggtggttccatcatcagcgaagacattattgtaactgctgctcattgcatgcaatcctacaaggcctaccaattcaaagtacgtttgggttccactgaatacgataatggtggtgaattggttgccgtcaagtctttcaaataccacgaaggttacaatcccgaaaccatggttaatgatgttgccgttatcaaattagccactccagtgcgtgaatcttccaaggtacgttatgttaaattggctgagaagacacctgctactggcaccccagctgtcgttactggttggggttctaagtgcttcttgttctgccaaactgcccctaaagttttgcaaaaggttgaggtcgatattgttgatgagaagacctgcgcttccagcgaatacaaatatggtgatgacatcaaggaaactatgttgtgtgcttatgctgttaagaaggatgcttgccaaggtgattctggtggtcctttggttgccaacaacaaattggtcggtgttgtttcctggggtaaaggttgtgcccttgctggctatcccggtgtatactgcgatgttgctactgtccgcagctggattgaaaagactgccaagagtttgtaa

SEQ ID NO: 7 - DNA, 717 bp, Lucilia sericata
ggcgctattcccaatgatttggatggccgcattgtcaatggtgtggataccaccattcaggcccatccctatcaggtttctttgcaaaccaacaatggtttccatttctgcggtggttccatcatcagcgaagacattattgtaactgctgctcattgcatgcaatcctacaaggcctaccaattcaaagtacgtttgggttccactgaatacgataatggtggtgaattggttgccgtcaagtctttcaaataccacgaaggttacaatcccgaaaccatggttaatgatgttgccgttatcaaattagccactccagtgcgtgaatcttccaaggtacgttatgttaaattggctgagaagacacctgctactggcaccccagctgtcgttactggttggggttctaagtgcttcttgttctgccaaactgcccctaaagttttgcaaaaggttgaggtcgatattgttgatgagaagacctgcgcttccagcgaatacaaatatggtgatgacatcaaggaaactatgttgtgtgcttatgctgttaagaaggatgcttgccaaggtgattctggtggtcctttggttgccaacaacaaattggtcggtgttgtttcctggggtaaaggttgtgcccttgctggctatcccggtgtatactgcgatgttgctactgtccgcagctggattgaaaagactgccaagagtttgtaa

SEQ ID NO: 8 - DNA, 687 bp, Lucilia sericata
attgtcaatggtgtggataccaccattcaggcccatccctatcaggtttctttgcaaaccaacaatggtttccatttctgcggtggttccatcatcagcgaagacattattgtaactgctgctcattgcatgcaatcctacaaggcctaccaattcaaagtacgtttgggttccactgaatacgataatggtggtgaattggttgccgtcaagtctttcaaataccacgaaggttacaatcccgaaaccatggttaatgatgttgccgttatcaaattagccactccagtgcgtgaatcttccaaggtacgttatgttaaattggctgagaagacacctgctactggcaccccagctgtcgttactggttggggttctaagtgcttcttgttctgccaaactgcccctaaagttttgcaaaaggttgaggtcgatattgttgatgagaagacctgcgcttccagcgaatacaaatatggtgatgacatcaaggaaactatgttgtgtgcttatgctgttaagaaggatgcttgccaaggtgattctggtggtcctttggttgccaacaacaaattggtcggtgttgtttcctggggtaaaggttgtgcccttgctggctatcccggtgtatactgcgatgttgctactgtccgcagctggattgaaaagactgccaagagtttgtaa

SEQ ID NO: 9 - protein, 60 aa, Artificial Sequence
  Aprotinin fused to EA-Tag
EARPDFCLEPPYTGPCKARIIRYFYNAKAGLCQTFVYGGCRAKRNNFKSAEDCMRTCGGA

SEQ ID NO: 10 - DNA, 183 bp, Artificial Sequence
  Aprotinin fused to GAAGCT-Tag
gaagctagaccagacttctgtttggaaccaccatacactggtccatgtaaggctagaatcatcagatacttctacaacgctaaggctggtttgtgtcagactttcgtttacggtggttgtagagctaagagaaacaacttcaagtccgctgaggactgtatgagaacttgtggtggtgcttaa

SEQ ID NO: 11 - DNA, 438 bp, Artificial Sequence
  Aprotinin sequence fused to sequence of the alpha mating factor from S. cerevisiae
atgagattcccatctattttcaccgctgtcttgttcgctgcctcctctgcattggctgcccctgttaacactaccactgaagacgagactgctcaaattccagctgaagcagttatcggttactctgaccttgagggtgatttcgacgtcgctgttttgcctttctctaactccactaacaacggtttgttgttcattaacaccactatcgcttccattgctgctaaggaagagggtgtctctctcgagaaaagagaagctagaccagacttctgtttggaaccaccatacactggtccatgtaaggctagaatcatcagatacttctacaacgctaaggctggtttgtgtcagactttcgtttacggtggttgtagagctaagagaaacaacttcaagtccgctgaggactgtatgagaacttgtggtggtgcttaa

SEQ ID NO: 12 - protein, 145 aa, Artificial Sequence
  Aprotinin sequence fused to sequence of the alpha mating factor from S. cerevisiae
MRFPSIFTAVLFAASSALAAPVNTTTEDETAQIPAEAVIGYSDLEGDFDVAVLPFSNSTNNGLLFINTTIASIAAKEEGVSLEKREARPDFCLEPPYTGPCKARIIRYFYNAKAGLCQTFVYGGCRAKRNNFKSAEDCMRTCGGA